European Patent Application EP 4 421 092 A1, published August 28, 2024. Title: ANTI-CD47-CLDN18.2 BISPECIFIC ANTIBODY AND USE THEREOF. Applicant: DRAGONBOAT BIOPHARMACEUTICAL (SHANGHAI) CO., LTD. SANYOU BIOPHARMACEUTICALS CO., LTD. The sequence listing filed with the application follows.

SEQUENCE LISTING (25 sequences)

SEQ ID NO: 1 - protein, 261 aa, Homo sapiens
MAVTACQGLGFVVSLIGIAGIIAATCMDQWSTQDLYNNPVTAVFNYQGLWRSCVRESSGFTECRGYFTLLGLPAMLQAVRALMIVGIVLGAIGLLVSIFALKCIRIGSMEDSAKANMTLTSGIMFIVSGLCAIAGVSVFANMLVTNFWMSTANMYTGMGGMVQTVQTRYTFGAALFVGWVAGGLTLIGGVMMCIACRGLAPEETNYKAVSYHASGHSVAYKPGGFKASTGFGSNTKNKKIYDGGARTEDEVQSYPSKHDYV

SEQ ID NO: 2 - protein, 330 aa, Artificial Sequence
  Human IgG1 heavy chain constant region
ASTKGPSVFPLAPSSKSTSGGTAALGCLVKDYFPEPVTVSWNSGALTSGVHTFPAVLQSSGLYSLSSVVTVPSSSLGTQTYICNVNHKPSNTKVDKKAEPKSCDKTHTCPPCPAPELLGGPSVFLFPPKPKDTLMISRTPEVTCVVVDVSHEDPEVKFNWYVDGVEVHNAKTKPREEQYNSTYRVVSVLTVLHQDWLNGKEYKCKVSNKALPAPIEKTISKAKGQPREPQVYTLPPSRDELTKNQVSLTCLVKGFYPSDIAVEWESNGQPENNYKTTPPVLDSDGSFFLYSKLTVDKSRWQQGNVFSCSVMHEALHNHYTQKSLSLSPGK

SEQ ID NO: 3 - protein, 107 aa, Artificial Sequence [sequence omitted]

SEQ ID NO: 4 - protein, 10 aa, Artificial Sequence
  A7H3L3-HCDR1
GFNIKDIYIY

SEQ ID NO: 5 - protein, 10 aa, Artificial Sequence
  A7H3L3-HCDR2
KIDPANGNTK

SEQ ID NO: 6 - protein, 8 aa, Artificial Sequence
  A7H3L3-HCDR3
GYGSGFAY

SEQ ID NO: 7 - protein, 11 aa, Artificial Sequence
  A7H3L3-LCDR1
RASQDISNHLN

SEQ ID NO: 8 - protein, 7 aa, Artificial Sequence
  A7H3L3-LCDR2
YTSRIHS

SEQ ID NO: 9 - protein, 9 aa, Artificial Sequence
  A7H3L3-LCDR3
QQGYTLPFT

SEQ ID NO: 10 - protein, 117 aa, Artificial Sequence
  A7H3L3-VH
QVQLVQSGAEVKKPGASVKVSCKASGFNIKDIYIYWVRQAPGQGLEWIGKIDPANGNTKYDQKFQGRATITADTSTNTAYLELSSLRSEDTAVYYCARGYGSGFAYWGQGTLVTVSS

SEQ ID NO: 11 - protein, 107 aa, Artificial Sequence
  A7H3L3-VL
DIQMTQSPSSLSASVGDRVTITCRASQDISNHLNWYQQKPGKAPKLLIYYTSRIHSGVPSSFRGSGSGTDYTLTISSLQPEDIATYFCQQGYTLPFTFGSGTKLEIK

SEQ ID NO: 12 - protein, 120 aa, Artificial Sequence
  NA3S-H1
QVQLVESGGGLVQPGGSLRLSCAASGSIFNIPVMGWYRQAPGKQRELVAGISTGGTTNYGDSVKGRFTISRDNAKNTVYLQMNSLKPEDTAVYYCNVLVVSGIGSTLEVWGQGTLVTVSS

SEQ ID NO: 13 - protein, 8 aa, Artificial Sequence
  NA3S-H1 CDR1
GSIFNIPV

SEQ ID NO: 14 - protein, 7 aa, Artificial Sequence
  NA3S-H1 CDR2
ISTGGTT

SEQ ID NO: 15 - protein, 14 aa, Artificial Sequence
  NA3S-H1 CDR3
NVLVVSGIGSTLEV

SEQ ID NO: 16 - protein, 577 aa, Artificial Sequence
  B8/B11 heavy chain
QVQLVESGGGLVQPGGSLRLSCAASGSIFNIPVMGWYRQAPGKQRELVAGISTGGTTNYGDSVKGRFTISRDNAKNTVYLQMNSLKPEDTAVYYCNVLVVSGIGSTLEVWGQGTLVTVSSGGGGSGGGGSQVQLVQSGAEVKKPGASVKVSCKASGFNIKDIYIYWVRQAPGQGLEWIGKIDPANGNTKYDQKFQGRATITADTSTNTAYLELSSLRSEDTAVYYCARGYGSGFAYWGQGTLVTVSSASTKGPSVFPLAPSSKSTSGGTAALGCLVKDYFPEPVTVSWNSGALTSGVHTFPAVLQSSGLYSLSSVVTVPSSSLGTQTYICNVNHKPSNTKVDKKAEPKSCDKTHTCPPCPAPELLGGPSVFLFPPKPKDTLMISRTPEVTCVVVDVSHEDPEVKFNWYVDGVEVHNAKTKPREEQYNSTYRVVSVLTVLHQDWLNGKEYKCKVSNKALPAPIEKTISKAKGQPREPQVYTLPPSRDELTKNQVSLTCLVKGFYPSDIAVEWESNGQPENNYKTTPPVLDSDGSFFLYSKLTVDKSRWQQGNVFSCSVMHEALHNHYTQKSLSLSPGK

SEQ ID NO: 17 - protein, 214 aa, Artificial Sequence
  B8/B10/B12 light chain
DIQMTQSPSSLSASVGDRVTITCRASQDISNHLNWYQQKPGKAPKLLIYYTSRIHSGVPSSFRGSGSGTDYTLTISSLQPEDIATYFCQQGYTLPFTFGSGTKLEIKRTVAAPSVFIFPPSDEQLKSGTASVVCLLNNFYPREAKVQWKVDNALQSGNSQESVTEQDSKDSTYSLSSTLTLSKADYEKHKVYACEVTHQGLSSPVTKSFNRGEC

SEQ ID NO: 18 - protein, 447 aa, Artificial Sequence
  B9 heavy chain
QVQLVQSGAEVKKPGASVKVSCKASGFNIKDIYIYWVRQAPGQGLEWIGKIDPANGNTKYDQKFQGRATITADTSTNTAYLELSSLRSEDTAVYYCARGYGSGFAYWGQGTLVTVSSASTKGPSVFPLAPSSKSTSGGTAALGCLVKDYFPEPVTVSWNSGALTSGVHTFPAVLQSSGLYSLSSVVTVPSSSLGTQTYICNVNHKPSNTKVDKKAEPKSCDKTHTCPPCPAPELLGGPSVFLFPPKPKDTLMISRTPEVTCVVVDVSHEDPEVKFNWYVDGVEVHNAKTKPREEQYNSTYRVVSVLTVLHQDWLNGKEYKCKVSNKALPAPIEKTISKAKGQPREPQVYTLPPSRDELTKNQVSLTCLVKGFYPSDIAVEWESNGQPENNYKTTPPVLDSDGSFFLYSKLTVDKSRWQQGNVFSCSVMHEALHNHYTQKSLSLSPGK

SEQ ID NO: 19 - protein, 344 aa, Artificial Sequence
  B9/B11 light chain
QVQLVESGGGLVQPGGSLRLSCAASGSIFNIPVMGWYRQAPGKQRELVAGISTGGTTNYGDSVKGRFTISRDNAKNTVYLQMNSLKPEDTAVYYCNVLVVSGIGSTLEVWGQGTLVTVSSGGGGSGGGGSDIQMTQSPSSLSASVGDRVTITCRASQDISNHLNWYQQKPGKAPKLLIYYTSRIHSGVPSSFRGSGSGTDYTLTISSLQPEDIATYFCQQGYTLPFTFGSGTKLEIKRTVAAPSVFIFPPSDEQLKSGTASVVCLLNNFYPREAKVQWKVDNALQSGNSQESVTEQDSKDSTYSLSSTLTLSKADYEKHKVYACEVTHQGLSSPVTKSFNRGEC

SEQ ID NO: 20 - protein, 577 aa, Artificial Sequence
  B10 heavy chain
QVQLVQSGAEVKKPGASVKVSCKASGFNIKDIYIYWVRQAPGQGLEWIGKIDPANGNTKYDQKFQGRATITADTSTNTAYLELSSLRSEDTAVYYCARGYGSGFAYWGQGTLVTVSSASTKGPSVFPLAPSSKSTSGGTAALGCLVKDYFPEPVTVSWNSGALTSGVHTFPAVLQSSGLYSLSSVVTVPSSSLGTQTYICNVNHKPSNTKVDKKAEPKSCDKTHTCPPCPAPELLGGPSVFLFPPKPKDTLMISRTPEVTCVVVDVSHEDPEVKFNWYVDGVEVHNAKTKPREEQYNSTYRVVSVLTVLHQDWLNGKEYKCKVSNKALPAPIEKTISKAKGQPREPQVYTLPPSRDELTKNQVSLTCLVKGFYPSDIAVEWESNGQPENNYKTTPPVLDSDGSFFLYSKLTVDKSRWQQGNVFSCSVMHEALHNHYTQKSLSLSPGKGGGGSGGGGSQVQLVESGGGLVQPGGSLRLSCAASGSIFNIPVMGWYRQAPGKQRELVAGISTGGTTNYGDSVKGRFTISRDNAKNTVYLQMNSLKPEDTAVYYCNVLVVSGIGSTLEVWGQGTLVTVSS

SEQ ID NO: 21 - protein, 572 aa, Artificial Sequence
  B12 heavy chain
QVQLVESGGGLVQPGGSLRLSCAASGSIFNIPVMGWYRQAPGKQRELVAGISTGGTTNYGDSVKGRFTISRDNAKNTVYLQMNSLKPEDTAVYYCNVLVVSGIGSTLEVWGQGTLVTVSSGGGGSQVQLVQSGAEVKKPGASVKVSCKASGFNIKDIYIYWVRQAPGQGLEWIGKIDPANGNTKYDQKFQGRATITADTSTNTAYLELSSLRSEDTAVYYCARGYGSGFAYWGQGTLVTVSSASTKGPSVFPLAPSSKSTSGGTAALGCLVKDYFPEPVTVSWNSGALTSGVHTFPAVLQSSGLYSLSSVVTVPSSSLGTQTYICNVNHKPSNTKVDKKAEPKSCDKTHTCPPCPAPELLGGPSVFLFPPKPKDTLMISRTPEVTCVVVDVSHEDPEVKFNWYVDGVEVHNAKTKPREEQYNSTYRVVSVLTVLHQDWLNGKEYKCKVSNKALPAPIEKTISKAKGQPREPQVYTLPPSRDELTKNQVSLTCLVKGFYPSDIAVEWESNGQPENNYKTTPPVLDSDGSFFLYSKLTVDKSRWQQGNVFSCSVMHEALHNHYTQKSLSLSPGK

SEQ ID NO: 22 - protein, 10 aa, Artificial Sequence
  Linker1
GGGGSGGGGS

SEQ ID NO: 23 - protein, 5 aa, Artificial Sequence
  Linker2
GGGGS

SEQ ID NO: 24 - protein, 452 aa, Artificial Sequence
  F4AM4-IgG1 heavy chain
QVQLVQSGAEVKKPGASVKMSCKASGYTFTSSVMHWVRQAPGQGLEWIGYINPYTDGTKYAQKFQGRATLTSDKSTSTAYMEFSSLRSEDTAVYYCGRPYYGTRYGSWFAYWGQGTLVTVSSASTKGPSVFPLAPSSKSTSGGTAALGCLVKDYFPEPVTVSWNSGALTSGVHTFPAVLQSSGLYSLSSVVTVPSSSLGTQTYICNVNHKPSNTKVDKKAEPKSCDKTHTCPPCPAPELLGGPSVFLFPPKPKDTLMISRTPEVTCVVVDVSHEDPEVKFNWYVDGVEVHNAKTKPREEQYNSTYRVVSVLTVLHQDWLNGKEYKCKVSNKALPAPIEKTISKAKGQPREPQVYTLPPSRDELTKNQVSLTCLVKGFYPSDIAVEWESNGQPENNYKTTPPVLDSDGSFFLYSKLTVDKSRWQQGNVFSCSVMHEALHNHYTQKSLSLSPGK

SEQ ID NO: 25 - protein, 214 aa, Artificial Sequence
  F4AM4-IgG1 light chain
DIQMTQSPSSLSASVGDRVTITCRASQDISNYLNWYQQKPGKAPKLLIYYTSRLHSGVPSRFSGSGSGTDYTLTISNLQPEDIATYYCQQGKNYPFTFGSGTKLEIKRTVAAPSVFIFPPSDEQLKSGTASVVCLLNNFYPREAKVQWKVDNALQSGNSQESVTEQDSKDSTYSLSSTLTLSKADYEKHKVYACEVTHQGLSSPVTKSFNRGEC